European Patent Application EP 4 190 904 A1, published June 7, 2023. Title: A microorganism producing L-valine and a method for producing L-valine using the same. Applicant: CJ CheilJedang Corporation. The sequence listing filed with the application follows.

SEQUENCE LISTING (50 sequences)

SEQ ID NO: 1 - protein, 613 aa, Unknown
  Corynebacterium sp. dihydroxy-acid dehydratase
MIPLRSKVTTVGRNAAGARALWRATGTKENEFGKPIVAIVNSYTQFVPGHVHLKNVGDIVADAVRKAGGVPKEFNTIAVDDGIAMGHGGMLYSLPSREIIADSVEYMVNAHTADAMVCISNCDKITPGMLNAAMRLNIPVVFVSGGPMEAGKAVVVDGVAHAPTDLITAISASASDAVDDAGLAAVEASACPTCGSCSGMFTANSMNCLTEALGLSLPGNGSTLATHAARRALFEKAGETVVELCRRYYGEEDESVLPRGIATKKAFENAMALDMAMGGSTNTILHILAAAQEGEVDFDLADIDELSKNVPCLSKVAPNSDYHMEDVHRAGGIPALLGELNRGGLLNKDVHSVHSNDLEGWLDDWDIRSGKTTEVATELFHAAPGGIRTTEAFSTENRWDELDTDAAKGCIRDVEHAYTADGGLVVLRGNISPDGAVIKSAGIEEELWNFTGPARVVESQEEAVSVILTKTIQAGEVLVVRYEGPSGGPGMQEMLHPTAFLKGSGLGKKCALITDGRFSGGSSGLSIGHVSPEAAHGGVIGLIENGDIVSIDVHNRKLEVQVSDEELQRRRDAMNASEKPWQPVNRNRVVTKALRAYAKMATSADKGAVRQVD

SEQ ID NO: 2 - protein, 383 aa, Unknown
  Corynebacterium sp. transaminase C
MKPSTRSNVQPFRVMQMLDRVHRRRREGKDTIMFCAGQPSTGAPEAVIEEAEIALRSGPLGYTEVIGDREFRERIADWHSATYDVDTNPDNVIVTTGSSGGFVASFIATLDHGDYVAMPTPGYPAYRNILESLGAKVLNLRCTAETRFQPTAQMLEELPHKPKAVIVTSPGNPTGTIIDPEELERIAKWCDDNDAVLISDEDYHGMSFGRPLATAHQFSKNAIVVGTLSKYFSMTGWRVGWIIVPDELVTSIENLQASLSLCAPAIGQAAGRAAFTLEAGAELDAHVEAYREAREVFVDKLPEIGLGTFADPDGGLYLWVDVSAYTDDSEEWVLRLLDEAGVAVAPGVDFDPEEGHKWIRLSLCASKEDTIEGVRKIGEFIKK

SEQ ID NO: 3 - protein, 922 aa, Unknown
  Corynebacterium sp. pyruvate dehydrogenase
MADQAKLGGKPSDDSNFAMIRDGVASYLNDSDPEETNEWMDSLDGLLQESSPERARYLMLRLLERASAKRVSLPPMTSTDYVNTIPTSMEPEFPGDEEMEKRYRRWIRWNAAIMVHRAQRPGIGVGGHISTYAGAAPLYEVGFNHFFRGKDHPGGGDQIFFQGHASPGMYARAFMEGRLSEDDLDGFRQEVSREQGGIPSYPHPHGMKDFWEFPTVSMGLGPMDAIYQARFNRYLENRGIKDTSDQHVWAFLGDGEMDEPESRGLIQQAALNNLDNLTFVVNCNLQRLDGPVRGNTKIIQELESFFRGAGWSVIKVVWGREWDELLEKDQDGALVEIMNNTSDGDYQTFKANDGAYVREHFFGRDPRTAKLVENMTDEEIWKLPRGGHDYRKVYAAYKRALETKDRPTVILAHTIKGYGLGHNFEGRNATHQMKKLTLDDLKLFRDKQGIPITDEQLEKDPYLPPYYHPGEDAPEIKYMKERRAALGGYLPERRENYDPIQVPPLDKLRSVRKGSGKQQIATTMATVRTFKELMRDKGLADRLVPIIPDEARTFGLDSWFPTLKIYNPHGQNYVPVDHDLMLSYREAPEGQILHEGINEAGSMASFIAAGTSYATHGKAMIPLYIFYSMFGFQRTGDSIWAAADQMARGFLLGATAGRTTLTGEGLQHMDGHSPVLASTNEGVETYDPSFAYEIAHLVHRGIDRMYGPGKGEDVIYYITIYNEPTPQPAEPEGLDVEGLHKGIYLYSRGEGTGHEANILASGVGMQWALKAASILEADYGVRANIYSATSWVNLARDGAARNKAQLRNPGADAGEAFVTTQLKQTSGPYVAVSDFSTDLPNQIREWVPGDYTVLGADGFGFSDTRPAARRFFNIDAESIVVAVLNSLAREGKIDVSVAAQAAEKFKLDDPTSVSVDPNAPEE

SEQ ID NO: 4 - protein, 437 aa, Unknown
  Corynebacterium sp. citrate synthase
MFERDIVATDNNKAVLHYPGGEFEMDIIEASEGNNGVVLGKMLSETGLITFDPGYVSTGSTESKITYIDGDAGILRYRGYDIADLAENATFNEVSYLLINGELPTPDELHKFNDEIRHHTLLDEDFKSQFNVFPRDAHPMATLASSVNILSTYYQDQLNPLDEAQLDKATVRLMAKVPMLAAYAHRARKGAPYMYPDNSLNARENFLRMMFGYPTEPYEIDPIMVKALDKLLILHADHEQNCSTSTVRMIGSAQANMFVSIAGGINALSGPLHGGANQAVLEMLEDIKNNHGGDATAFMNKVKNKEDGVRLMGFGHRVYKNYDPRAAIVKETAHEILEHLGGDDLLDLAIKLEEIALADDYFISRKLYPNVDFYTGLIYRAMGFPTDFFTVLFAIGRLPGWIAHYREQLGAADNKINRPRQVYTGNESRKLVPREER

SEQ ID NO: 5 - protein, 922 aa, Unknown
  Corynebacterium sp. pyruvate dehydrogenase variant
MADQAKLGGKPSDDSNFAMIRDGVASYLNDSDPEETNEWMDSLDGLLQESSPERARYLMLRLLERASAKRVSLPPMTSTDYVNTIPTSMEPEFPGDEEMEKRYRRWIRWNAAIMVHRAQRPGIGVGGHISTYAGAAPLYEVGFNHFFRGKDHPGGGDQIFFQGHASPGMYARAFMEGRLSEDDLDGFRQEVSREQGGIPSYPHPHGMKDFWEFPTVSMGLGPMDAIYQARFNRYLENRGIKDTSDQHVWAFLGDGEMDEPESRGLIQQAALNNLDNLTFVVNCNLQRLDGPVRGNTKIIQELESFFRGAGWSVIKVVWGREWDELLEKDQDGALVEIMNNTSDGDYQTFKANDGAYVREHFFGRDPRTAKLVENMTDEEIWKLPRGGHDYRKVYAAYKRALETKDRPTVILAHTIKGYGLGHNFEGRNATHAMKKLTLDDLKLFRDKQGIPITDEQLEKDPYLPPYYHPGEDAPEIKYMKERRAALGGYLPERRENYDPIQVPPLDKLRSVRKGSGKQQIATTMATVRTFKELMRDKGLADRLVPIIPDEARTFGLDSWFPTLKIYNPHGQNYVPVDHDLMLSYREAPEGQILHEGINEAGSMASFIAAGTSYATHGKAMIPLYIFYSMFGFQRTGDSIWAAADQMARGFLLGATAGRTTLTGEGLQHMDGHSPVLASTNEGVETYDPSFAYEIAHLVHRGIDRMYGPGKGEDVIYYITIYNEPTPQPAEPEGLDVEGLHKGIYLYSRGEGTGHEANILASGVGMQWALKAASILEADYGVRANIYSATSWVNLARDGAARNKAQLRNPGADAGEAFVTTQLKQTSGPYVAVSDFSTDLPNQIREWVPGDYTVLGADGFGFSDTRPAARRFFNIDAESIVVAVLNSLAREGKIDVSVAAQAAEKFKLDDPTSVSVDPNAPEE

SEQ ID NO: 6 - protein, 922 aa, Unknown
  Corynebacterium sp. pyruvate dehydrogenase variant
MADQAKLGGKPSDDSNFAMIRDGVASYLNDSDPEETNEWMDSLDGLLQESSPERARYLMLRLLERASAKRVSLPPMTSTDYVNTIPTSMEPEFPGDEEMEKRYRRWIRWNAAIMVHRAQRPGIGVGGHISTYAGAAPLYEVGFNHFFRGKDHPGGGDQIFFQGHASPGMYARAFMEGRLSEDDLDGFRQEVSREQGGIPSYPHPHGMKDFWEFPTVSMGLGPMDAIYQARFNRYLENRGIKDTSDQHVWAFLGDGEMDEPESRGLIQQAALNNLDNLTFVVNCNLQRLDGPVRGNTKIIQELESFFRGAGWSVIKVVWGREWDELLEKDQDGALVEIMNNTSDGDYQTFKANDGAYVREHFFGRDPRTAKLVENMTDEEIWKLPRGGHDYRKVYAAYKRALETKDRPTVILAHTIKGYGLGHNFEGRNATHQMKALTLDDLKLFRDKQGIPITDEQLEKDPYLPPYYHPGEDAPEIKYMKERRAALGGYLPERRENYDPIQVPPLDKLRSVRKGSGKQQIATTMATVRTFKELMRDKGLADRLVPIIPDEARTFGLDSWFPTLKIYNPHGQNYVPVDHDLMLSYREAPEGQILHEGINEAGSMASFIAAGTSYATHGKAMIPLYIFYSMFGFQRTGDSIWAAADQMARGFLLGATAGRTTLTGEGLQHMDGHSPVLASTNEGVETYDPSFAYEIAHLVHRGIDRMYGPGKGEDVIYYITIYNEPTPQPAEPEGLDVEGLHKGIYLYSRGEGTGHEANILASGVGMQWALKAASILEADYGVRANIYSATSWVNLARDGAARNKAQLRNPGADAGEAFVTTQLKQTSGPYVAVSDFSTDLPNQIREWVPGDYTVLGADGFGFSDTRPAARRFFNIDAESIVVAVLNSLAREGKIDVSVAAQAAEKFKLDDPTSVSVDPNAPEE

SEQ ID NO: 7 - protein, 922 aa, Unknown; identical to SEQ ID NO: 6
  Corynebacterium sp. citrate synthase variant

SEQ ID NO: 8 - protein, 437 aa, Unknown
  Corynebacterium sp. citrate synthase variant
MFERDIVATDNNKAVLHYPGGEFEMDIIEASEGNNGVVLGKMLSETGLITFDPGYVSTGSTESKITYIDGDAGILRYRGYDIADLAENATFNEVSYLLINGELPTPDELHKFNDEIRHHTLLDEDFKSQFNVFPRDAHPMATLASSVNILSTYYQDQLNPLDEAQLDKATVRLMAKVPMLAAYAHRARKGAPYMYPDNSLNARENFLRMMFGYPTEPYEIDPIMVKALDKLLILHADHEQNCSTSTVRMIGSAQANMFVSIAGGINALSGPLHGGANQAVLEMLEDIKNNHGGDATAFMNKVKNKEDGVRLIGFGHRVYKNYDPRAAIVKETAHEILEHLGGDDLLDLAIKLEEIALADDYFISRKLYPNVDFYTGLIYRAMGFPTDFFTVLFAIGRLPGWIAHYREQLGAADNKINRPRQVYTGNESRKLVPREER

SEQ ID NO: 9 - DNA, 32 bp, Artificial Sequence
  primer
aatttctagaggcagaccctattctatgaagg

SEQ ID NO: 10 - DNA, 30 bp, Artificial Sequence
  primer
agtgtttcggtctttacagacacgagggac

SEQ ID NO: 11 - DNA, 30 bp, Artificial Sequence
  primer
gtccctcgtgtctgtaaagaccgaaacact

SEQ ID NO: 12 - DNA, 32 bp, Artificial Sequence
  primer
aatttctagacgtgggagtgtcactcgcttgg

SEQ ID NO: 13 - DNA, 41 bp, Artificial Sequence
  primer
ttcgagctcggtacccggtctagagcactttcgctcgcacc

SEQ ID NO: 14 - DNA, 36 bp, Artificial Sequence
  primer
gatttgaaaagcgcatcagaaacatcccagcgctac

SEQ ID NO: 15 - DNA, 36 bp, Artificial Sequence
  primer
gtagcgctgggatgtttctgatgcgcttttcaaatc

SEQ ID NO: 16 - DNA, 41 bp, Artificial Sequence
  primer
gaaacactatgatcccacttcgttcaaaagtcaccaccgtc

SEQ ID NO: 17 - DNA, 41 bp, Artificial Sequence
  primer
gacggtggtgacttttgaacgaagtgggatcatagtgtttc

SEQ ID NO: 18 - DNA, 41 bp, Artificial Sequence
  primer
gcatgcctgcaggtcgactctagagcgtgtgcaacgccgtc

SEQ ID NO: 19 - DNA, 50 bp, Artificial Sequence
  primer
gctcggtacccggggatcctctagaccgcttccttggctgcctgaagatg

SEQ ID NO: 20 - DNA, 26 bp, Artificial Sequence
  primer
tgcttggcttcacaagagacaagcct

SEQ ID NO: 21 - DNA, 26 bp, Artificial Sequence
  primer
aggcttgtctcttgtgaagccaagca

SEQ ID NO: 22 - DNA, 50 bp, Artificial Sequence
  primer
gcctgcaggtcgacctagatctagacctcatcagagataagaacagcatc

SEQ ID NO: 23 - DNA, 50 bp, Artificial Sequence
  primer
gctcggtacccggggatcctctagatactccggtctgctttatgcaggta

SEQ ID NO: 24 - DNA, 36 bp, Artificial Sequence
  primer
aactaacctagtcgcttaagagacaagcctatctgc

SEQ ID NO: 25 - DNA, 36 bp, Artificial Sequence
  primer
gcagataggcttgtctcttaagcgactaggttagtt

SEQ ID NO: 26 - DNA, 50 bp, Artificial Sequence
  primer
gcctgcaggtcgacctagatctagaaagtgccacgagcatttcatcagct

SEQ ID NO: 27 - DNA, 50 bp, Artificial Sequence
  primer
gctcggtacccggggatcctctagataccgtccaaccggtactttgaacc

SEQ ID NO: 28 - DNA, 20 bp, Artificial Sequence
  primer
ttgatcggccacttccacac

SEQ ID NO: 29 - DNA, 21 bp, Artificial Sequence
  primer
ggtgtggaagtggccgatcaa

SEQ ID NO: 30 - DNA, 50 bp, Artificial Sequence
  primer
gcctgcaggtcgacctagatctagagatcgtcttcagaaaggcgaccctc

SEQ ID NO: 31 - DNA, 50 bp, Artificial Sequence
  primer
gctcggtacccggggatcctctagaaccgtggcatcaaggacacctctga

SEQ ID NO: 32 - DNA, 22 bp, Artificial Sequence
  primer
agcttcttcattgcgtgggttg

SEQ ID NO: 33 - DNA, 22 bp, Artificial Sequence
  primer
caacccacgcaatgaagaagct

SEQ ID NO: 34 - DNA, 21 bp, Artificial Sequence
  primer
aagcgtcagtgccttcatctg

SEQ ID NO: 35 - DNA, 22 bp, Artificial Sequence
  primer
ccagatgaaggcactgacgctt

SEQ ID NO: 36 - DNA, 50 bp, Artificial Sequence
  primer
gcctgcaggtcgacctagatctagaagatggagtcaccggtgcgctggaa

SEQ ID NO: 37 - DNA, 50 bp, Artificial Sequence
  primer
gctcggtacccggggatcctctagaacctttccctggaattttttccttt

SEQ ID NO: 38 - DNA, 38 bp, Artificial Sequence
  primer
tgtcccttgaggtgatttccacacctcctgttggaatg

SEQ ID NO: 39 - DNA, 37 bp, Artificial Sequence
  primer
tccaacaggaggtgtggaaatcacctcaagggacaga

SEQ ID NO: 40 - DNA, 50 bp, Artificial Sequence
  primer
gcctgcaggtcgacctagatctagatgctgcgcggcaagcgccgtggatt

SEQ ID NO: 41 - DNA, 50 bp, Artificial Sequence
  primer
gctcggtacccggggatcctctagaaccctgaagctgtcagttcctagca

SEQ ID NO: 42 - DNA, 21 bp, Artificial Sequence
  primer
ccctttcaaacacatttgttc

SEQ ID NO: 43 - DNA, 22 bp, Artificial Sequence
  primer
cgaacaaatgtgtttgaaaggg

SEQ ID NO: 44 - DNA, 50 bp, Artificial Sequence
  primer
gcctgcaggtcgacctagatctagatgcgcggtgtgcgtacgcagccagc

SEQ ID NO: 45 - DNA, 50 bp, Artificial Sequence
  primer
gctcggtacccggggatcctctagatatgtgagcactggctctaccgagt

SEQ ID NO: 46 - DNA, 22 bp, Artificial Sequence
  primer
aggtggagcaggtctgctcgtg

SEQ ID NO: 47 - DNA, 22 bp, Artificial Sequence
  primer
cacgagcagacctgctccacct

SEQ ID NO: 48 - DNA, 23 bp, Artificial Sequence
  primer
tgtccgaagccgatgaggcggac

SEQ ID NO: 49 - DNA, 24 bp, Artificial Sequence
  primer
cgtccgcctcatcggcttcggaca

SEQ ID NO: 50 - DNA, 50 bp, Artificial Sequence
  primer
gcctgcaggtcgacctagatctagagtcagagattacgagatcttccggt